European Patent Application EP 4 803 534 A1, published September 9, 2026. Title: 突变的br2蛋白及其应用. Applicant: 山东舜丰生物科技有限公司. Application CN. The sequence listing filed with the application follows.

SEQUENCE LISTING (6 sequences)

SEQ ID NO: 1 - RNA, 4137 nt, synthetic construct
  source 1..4137: mol_type = other RNA
  misc_feature 1..4137: note = CDS
atgtctagcagcgacccggaggagatcagggcgcgcgtcgtcgttctcggttcgccccatgccgacggcggcgacgagtgggcccggcccgagctcgaggccttccatctgccgtctcccgcccaccagcctcctggcttcctagccgggcaaccggaagcagcagagcaacccacgctccctgctcctgctggccgcagcagcagcagcaacacgcctactacatctggcggtggcggcgctgctcctcctcttccttcttcgcctccccctccgccggcttctctggagaccgagcagccgcccaatgccaggccagcctccgccggcgccaatgacagcaagaagcccaccccgcccgccgccctgcgcgacctcttccgcttcgccgacggcctcgactgcgcgctcatgctcatcggcaccctcggcgcgctcgtccacggctgctcgctccccgtcttcctccgcttcttcgccgacctcgtcgactccttcggctcccacgccgacgacccggacaccatggtccgcctcgtcgtcaagtacgccttctacttcctcgtcgtcggagcggcaatctgggcatcctcgtgggcagagatctcttgctggatgtggaccggcgagcggcagtcgacgcggatgcggatccggtacctggacgcggcgctgcggcaggacgtgtccttcttcgacaccgacgtgcgggcctcggacgtgatctacgccatcaacgcggacgccgtggtggtgcaggacgccatcagcgagaagctgggcaacctcatccactacatggccaccttcgtggccggcttcgtcgtggggttcacggccgcgtggcagctggcgctggtcacgctggccgtggtgccgctcatcgccgtcatcggtgggctgagcgccgccgcgctcgccaagctctcgtcccgcagccaggacgcgctctcgggcgccagcggcatcgcggagcaggcgctcgcgcagatacggatcgtgcaggcgttcgtcggcgaggagcgcgagatgcgggcctactcggcggcgctggccgtggcgcagaggatcggctaccgcagcggcttcgccaaggggctcggcctcggcggcacctacttcaccgtcttctgctgctacgggctcctgctctggtacggcggccacctcgtgcgcgcccagcacaccaacggcgggctcgccatcgccaccatgttctccgtcatgatcggcggactggccctcgggcagtcggcgccgagcatggccgcgttcgccaaggcgcgtgtggcggctgccaagatcttccgcatcatcgaccacaggccgggcatctcctcgcgcgacggcgcggagccggagtcggtgacggggcgggtggagatgcggggcgtggacttcgcgtacccgtcgcggccggacgtccccatcctgcgcggcttctcgctgagcgtgcccgccgggaagaccatcgcgctggtgggcagctccggctccgggaagagcacggtggtgtcgctcatcgagagattctacgaccccagcgcagggcaaatcctgctggacgggcacgacctcaggtcgctgaagctgcggtggctgcggcggcagatcgggctggtgagccaggagccggcgctgttcgcgacgagcatcagggagaacctgctgctggggcgggacagccagagcgcgacgctggcggagatggaggaggcggccagggtggccaacgcccactccttcatcatcaaactccccgacggctacgacacgcaggttggggagcgcggcctgcagctctccggtggccagaagcagcgcatcgccatcgcccgcgccatgctcaagaaccccgccatcctgctgctggacgaggccaccagcgcgctggactccgagtctgagaagctcgtgcaggaggcgctggaccgcttcatgatcgggcgcaccaccctggtgatcgcgcacaggctgtccaccatccgcaaggccgacgtggtggccgtgctgcagggcggcgccgtctccgagatgggcgcgcacgacgagctgatggccaagggcgagaacggcacctacgccaagctcatccgcatgcaggagcaggcgcacgaggcggcgctcgtcaacgcccgccgcagcagcgccaggccctccagcgcccgcaactccgtcagctcgcccatcatgacgcgcaactcctcctacggccgctccccctactcccgccgcctctccgacttctccacctccgacttcaccctctccatccacgacccgcaccaccaccaccggaccatggcggacaagcagctggcgttccgcgccggcgccagctccttcctgcgcctcgccaggatgaactcgcccgagtgggcctacgcgctcgccggctccatcggctccatggtctgcggctccttcagcgccatcttcgcctacatcctcagcgccgtgctcagcgtgtactacgcgccggacccgcggtacatgaagcgcgagatcgccaaatactgctacctgctcatcggcatgtcctccgcggcgctgctgttcaacacggtgcagcacgtgttctgggacacggtgggcgagaacctgaccaagcgggtgcgcgagaagatgttcgccgccgtgctccgcaacgagatcgcctggttcgacgcggacgagaacgccagcgcgcgcgtggccgccaggctcgcgctggacgcccagaacgtgcgctccgccatcggggaccgcatctccgtcatcgtccagaactcggcgctgatgctggtggcctgcaccgcggggttcgtcctccagtggcgcctcgcgctcgtgctcctcgccgtgttcccgctcgtcgtgggcgccaccgtgctgcagaagatgttcatgaagggcttctcgggggacctggaggccgcgcacgccagggcgacgcagatcgcgggcgaggccgtggccaacctgcgcaccgtggccgcgttcaacgcggagcgcaagatcacggggctgttcgaggccaacctgcgcggcccgctccggcgctgcttctggaaggggcagatcgccggcagcggctacggcgtggcgcagttcctgctgtacgcgtcctacgcgctggggctgtggtacgcggcgtggctggtgaagcacggcgtgtccgacttctcgcgcaccatccgcgtgttcatggtgctgatggtgtccgcgaacggcgccgccgagacgctgacgctggcgccggacttcatcaagggcgggcgcgcgatgcggtcggtgttcgagacgatcgaccgcaagacggaggtggagcccgacgacgtggacgcggcgccggtgccggagcggccgaggggcgaggtggagctgaagcacgtggacttctcgtacccgtcgcggccggacatccaggtgttccgcgacctgagcctccgtgcgcgcgccgggaagacgctggcgctggtggggccgagcgggtgcggcaagagctcggtgctggctctggtgcagcggttctacgagcccacgtccgggcgcgtgctcctggacggcaaggacgtgcgcaagtacaacctgcgggcgctgcggcgcgtggtggcggtggtgccgcaggagccgttcctgttcgcggcgagcatccacgagaacatcgcgtacgggcgcgagggcgcgacggaggcggaggtggtggaggcggcggcgcaggcgaacgcgcaccggttcatcgcggcgctgccggaggggtaccggacgcaggtgggcgagcgcggggtgcagctgtcgggagggcagcggcagcggatcgcgatcgcgcgcgcgctagtgaagcaggcggccatcgtgctgctggacgaggcgaccagcgcgctggacgccgagtcggagcggtgcgtgcaggaggcgctggagcgcgcggggtccgggcgcaccaccatcgtggtggcgcaccggctggccacggtgcgcggcgcgcacaccatcgcggtcatcgacgacggcaaggtggcggagcaggggtcgcactcgcacctgctcaagcaccatcccgacgggtgctacgcgcggatgctgcagctgcagcggctgacgggcgcggcggccgggcccgggccgtcgtcctcgtgcaacggggccgcgtag

SEQ ID NO: 2 - RNA, 368 nt, synthetic construct
  source 1..368: mol_type = other RNA
  misc_feature 1..368: note = 3 UTR
gacggaatggatgggtttggttcctcgagagattgatgggtgaggaagctgaagctccgggatcaaatggtggtactccatgatcgcaacaatgagggggaaaaaaagaaaggagaaaatacggtggttcatatgattgtacaatttgacgatctgtttgagtcggggttttaggatgatgtaaaccttcactcgccttttttttactcttgtttctcatccgcatcagtatcatctatctacatacagtgtcagagatgggaactgatccgcatcatcatctacctcccaaggcaccccatattgtattaatgtacttagttagcctgttttatatatacttataagtaccaaatagcagaatttta

SEQ ID NO: 3 - protein, 1378 aa, unidentified
  REGION 1..1378: note = br2
MSSSDPEEIRARVVVLGSPHADGGDEWARPELEAFHLPSPAHQPPGFLAGQPEAAEQPTLPAPAGRSSSSNTPTTSGGGGAAPPLPSSPPPPPASLETEQPPNARPASAGANDSKKPTPPAALRDLFRFADGLDCALMLIGTLGALVHGCSLPVFLRFFADLVDSFGSHADDPDTMVRLVVKYAFYFLVVGAAIWASSWAEISCWMWTGERQSTRMRIRYLDAALRQDVSFFDTDVRASDVIYAINADAVVVQDAISEKLGNLIHYMATFVAGFVVGFTAAWQLALVTLAVVPLIAVIGGLSAAALAKLSSRSQDALSGASGIAEQALAQIRIVQAFVVEEREMRAYSAALAVAQRIGYRSGFAKGLGLGGTYFTVFCCYGLLLWYGGHLVRAQHTNGGLAIATMFSVMIGGLALGQSAPSMAAFAKARVAAAKIFRIIDHRPGISSRDGAEPESVTGRVEMRGVDFAYPSRPDVPILRGFSLSVPAGKTIALVGSSGSGKSTVVSLIERFYDPSAGQILLDGHDLRSLKLRWLRRQIGLVSQEPALFATSIRENLLLGRDSQSATLAEMEEAARVANAHSFIIKLPDGYDTQVGERGLQLSGGQKQRIAIARAMLKNPAILLLDEATSALDSESEKLVQEALDRFMIGRTTLVIAHRLSTIRKADVVAVLQGGAVSEMGAHDELMAKGENGTYAKLIRMQEQAHEAALVNARRSSARPSSARNSVSSPIMTRNSSYGRSPYSRRLSDFSTSDFTLSIHDPHHHHRTMADKQLAFRAGASSFLRLARMNSPEWAYALAGSIGSMVCGSFSAIFAYILSAVLSVYYAPDPRYMKREIAKYCYLLIGMSSAALLFNTVQHVFWDTVGENLTKRVREKMFAAVLRNEIAWFDADENASARVAARLALDAQNVRSAIGDRISVIVQNSALMLVACTAGFVLQWRLALVLLAVFPLVVGATVLQKMFMKGFSGDLEAAHARATQIAGEAVANLRTVAAFNAERKITGLFEANLRGPLRRCFWKGQIAGSGYGVAQFLLYASYALGLWYAAWLVKHGVSDFSRTIRVFMVLMVSANGAAETLTLAPDFIKGGRAMRSVFETIDRKTEVEPDDVDAAPVPERPRGEVELKHVDFSYPSRPDIQVFRDLSLRARAGKTLALVGPSGCGKSSVLALVQRFYEPTSGRVLLDGKDVRKYNLRALRRVVAVVPQEPFLFAASIHENIAYGREGATEAEVVEAAAQANAHRFIAALPEGYRTQVGERGVQLSGGQRQRIAIARALVKQAAIVLLDEATSALDAESERCVQEALERAGSGRTTIVVAHRLATVRGAHTIAVIDDGKVAEQGSHSHLLKHHPDGCYARMLQLQRLTGAAAGPGPSSSCNGAA

SEQ ID NO: 4 - protein, 1045 aa, synthetic construct
  REGION 1..1045: note = Cas12i
MKKVEVSRPYQSLLLPNHRKFKYLDETWNAYKSVKSLLHRFLVCAYGAVPFNKFVEVVEKVDNDQLVLAFAVRLFRLVPVESTSFAKVDKANLAKSLANHLPVGTAIPANVQSYFDSNFDPKKYMWIDCAWEADRLAREMGLSASQFSEYATTMLWEDWLPLNKDDVNGWGSVSGLFGEGKKEDRQQKVKMLNNLLNGIKKNPPKDYTQYLKILLNAFDAKSHKEAVKNYKGDSTGRTASYLSEKSGEITELMLEQLMSNIQRDIGDKQKEISLPKKDVVKKYLESESGVPYDQNLWSQAYRNAASSIKKTDTRNFNSTLEKFKNEVELRGLLSEGDDVEILRSKFFSSEFHKTPDKFVIKPEHIGFNNKYNVVAELYKLKAEATDFESAFATVKDEFEEKGIKHPIKNILEYIWNNEVPVEKWGRVARFNQSEEKLLRIKANPTVECNQGMTFGNSAMVGEVLRSNYVSKKGALVSGEHGGRLIGQNNMIWLEMRLLNKGKWETHHVPTHNMKFFEEVHAYNPSLADSVNVRNRLYRSEDYTQLPSSITDGLKGNPKAKLLKRQHCALNNMTANVLNPKLSFTINKKNDDYTVIIVHSVEVSKPRREVLVGDYLVGMDQNQTASNTYAVMQVVKPKSTDAIPFRNMWVRFVESGSIESRTLNSRGEYVDQLNHDGVDLFEIGDTEWVDSARKFFNKLGVKHKDGTLVDLSTAPRKAYAFNNFYFKTMLNHLRSNEVDLTLLRNEILRVANGRFSPMRLGSLSWTTLKALGSFKSLVLSYFDRLGAKEMVDKEAKDKSLFDLLVAINNKRSNKREERTSRIASSLMTVAQKYKVDNAVVHVVVEGNLSSTDRSASKAHNRNTMDWCSRAVVKKLEDMCNLYGFNIKGVPAFYTSHQDPLVHRADYDDPKPALRCRYSSYSRADFSKWGQNALAAVVRWASNKKSNTCYKVGAVEFLKQHGLFADKKLTVEQFLSKVKDEEILIPRRGGRVFLTTHRLLAESTFVYLNGVKYHSCNADEVAAVNICLNDWVIPCKKKMKEESSASG

SEQ ID NO: 5 - RNA, 4101 nt, synthetic construct
  source 1..4101: mol_type = other RNA
  misc_feature 1..4101: note = CDS
atgtctagcagcgacccggaggagatcagggcgcgcgtcgtcgttctcggttcgccccatgccgacggcggcgacgagtgggcccggcccgagctcgaggccttccatctgccgtctcccgcccaccagcctcctggcttcctagccgggcaaccggaagcagcagagcaacccacgctccctgctcctgctggccgcagcagcagcagcaacacgcctactacatctggcggtggcggcgctgctcctcctcttccttcttcgcctccccctccgccggcttctctggagaccgagcagccgcccaatgccaggccagcctccgccggcgccaatgacagcaagaagcccaccccgcccgccgccctgcgcgacctcttccgcttcgccgacggcctcgactgcgcgctcatgctcatcggcaccctcggcgcgctcgtccacggctgctcgctccccgtcttcctccgcttcttcgccgacctcgtcgactccttcggctcccacgccgacgacccggacaccatggtccgcctcgtcgtcaagtacgccttctacttcctcgtcgtcggagcggcaatctgggcatcctcgtgggcagagatctcttgctggatgtggaccggcgagcggcagtcgacgcggatgcggatccggtacctggacgcggcgctgcggcaggacgtgtccttcttcgacaccgacgtgcgggcctcggacgtgatctacgccatcaacgcggacgccgtggtggtgcaggacgccatcagcgagaagctgggcaacctcatccactacatggccaccttcgtggccggcttcgtcgtggggttcacggccgcgtggcagctggcgctggtcacgctggccgtggtgccgctcatcgccgtcatcggtgggctgagcgccgccgcgctcgccaagctctcgtcccgcagccaggacgcgctctcgggcgccagcggcatcgcggagcaggcgctcgcgcagatacggatcgtgcaggcgttcgtcggcgaggagcgcgagatgcgggcctactcggcggcgctggccgtggcgcagaggatcggctaccgcagcggcttcgccaaggggctcggcctcggcggcacctacttcaccgtcttctgctgctacgggctcctgctctggtacggcggccacctcgtgcgcgcccagcacaccaacggcgggctcgccatcgccaccatgttctccgtcatgatcggcggactggccctcgggcagtcggcgccgagcatggccgcgttcgccaaggcgcgtgtggcggctgccaagatcttccgcatcatcgaccacaggccgggcatctcctcgcgcgacggcgcggagccggagtcggtgacggggcgggtggagatgcggggcgtggacttcgcgtacccgtcgcggccggacgtccccatcctgcgcggcttctcgctgagcgtgcccgccgggaagaccatcgcgctggtgggcagctccggctccgggaagagcacggtggtgtcgctcatcgagagattctacgaccccagcgcagggcaaatcctgctggacgggcacgacctcaggtcgctgaagctgcggtggctgcggcggcagatcgggctggtgagccaggagccggcgctgttcgcgacgagcatcagggagaacctgctgctggggcgggacagccagagcgcgacgctggcggagatggaggaggcggccagggtggccaacgcccactccttcatcatcaaactccccgacggctacgacacgcaggttggggagcgcggcctgcagctctccggtggccagaagcagcgcatcgccatcgcccgcgccatgctcaagaaccccgccatcctgctgctggacgaggccaccagcgcgctggactccgagtctgagaagctcgtgcaggaggcgctggaccgcttcatgatcgggcgcaccaccctggtgatcgcgcacaggctgtccaccatccgcaaggccgacgtggtggccgtgctgcagggcggcgccgtctccgagatgggcgcgcacgacgagctgatggccaagggcgagaacggcacctacgccaagctcatccgcatgcaggagcaggcgcacgaggcggcgctcgtcaacgcccgccgcagcagcgccaggccctccagcgcccgcaactccgtcagctcgcccatcatgacgcgcaactcctcctacggccgctccccctactcccgccgcctctccgacttctccacctccgacttcaccctctccatccacgacccgcaccaccaccaccggaccatggcggacaagcagctggcgttccgcgccggcgccagctccttcctgcgcctcgccaggatgaactcgcccgagtgggcctacgcgctcgccggctccatcggctccatggtctgcggctccttcagcgccatcttcgcctacatcctcagcgccgtgctcagcgtgtactacgcgccggacccgcggtacatgaagcgcgagatcgccaaatactgctacctgctcatcggcatgtcctccgcggcgctgctgttcaacacggtgcagcacgtgttctgggacacggtgggcgagaacctgaccaagcgggtgcgcgagaagatgttcgccgccgtgctccgcaacgagatcgcctggttcgacgcggacgagaacgccagcgcgcgcgtggccgccaggctcgcgctggacgcccagaacgtgcgctccgccatcggggaccgcatctccgtcatcgtccagaactcggcgctgatgctggtggcctgcaccgcggggttcgtcctccagtggcgcctcgcgctcgtgctcctcgccgtgttcccgctcgtcgtgggcgccaccgtgctgcagaagatgttcatgaagggcttctcgggggacctggaggccgcgcacgccagggcgacgcagatcgcgggcgaggccgtggccaacctgcgcaccgtggccgcgttcaacgcggagcgcaagatcacggggctgttcgaggccaacctgcgcggcccgctccggcgctgcttctggaaggggcagatcgccggcagcggctacggcgtggcgcagttcctgctgtacgcgtcctacgcgctggggctgtggtacgcggcgtggctggtgaagcacggcgtgtccgacttctcgcgcaccatccgcgtgttcatggtgctgatggtgtccgcgaacggcgccgccgagacgctgacgctggcgccggacttcatcaagggcgggcgcgcgatgcggtcggtgttcgagacgatcgaccgcaagacggaggtggagcccgacgacgtggacgcggcgccggtgccggagcggccgaggggcgaggtggagctgaagcacgtggacttctcgtacccgtcgcggccggacatccaggtgttccgcgacctgagcctccgtgcgcgcgccgggaagacgctggcgctggtggggccgagcgggtgcggcaagagctcggtgctggctctggtgcagcggttctacgagcccacgtccgggcgcgtgctcctggacggcaaggacgtgcgcaagtacaacctgcgggcgctgcggcgcgtggtggcggtggtgccgcaggagccgttcctgttcgcggcgagcatccacgagaacatcgcgtacgggcgcgagggcgcgacggaggcggaggtggtggaggcggcggcgcaggcgaacgcgcaccggttcatcgcggcgctgccggaggggtaccggacgcaggtgggcgagcgcggggtgcagctgtcgggagggcagcggcagcggatcgcgatcgcgcgcgcgctagtgaagcaggcggccatcgtgctgctggacgaggcgaccagcgcgctggacgccgagtcggagcggtgcgtgcaggaggcgctggagcgcgcggggtccgggcgcaccaccatcgtggtggcgcaccggctggccacggtgcgcggcgcgcacaccatcgcggtcatcgacgacggcaaggtggcggagcaggggtcgcactcgcacctgctcaagcaccatcccgacgggtgctacgcgcggatgctgcagctgcagcggctgacgggcgcggcggccggg

SEQ ID NO: 6 - RNA, 329 nt, synthetic construct
  source 1..329: mol_type = other RNA
  misc_feature 1..329: note = 3 UTR
tgggtgaggaagctgaagctccgggatcaaatggtggtactccatgatcgcaacaatgagggggaaaaaaagaaaggagaaaatacggtggttcatatgattgtacaatttgacgatctgttttcggggttttaggatgatgtaaaccttcactcgccttttttttactcttgtttctcatccgcatcagtatcatctatctacatacagtgtcagagatgggaactgatccgcatcatcatctacctcccaaggcaccccatattgtattaatgtacttagttagcctgttttatatatacttataagtaccaaatagcagaatttta